European Patent Specification EP 3 615 005 B1, published July 30, 2025. Title: Compositions and Methods for Vaccine Delivery. Applicant: The Henry M. Jackson Foundation for the Advancement of Miliary Medicine, Inc. Application PCT/US18/29906. The sequence listing filed with the application follows.

SEQUENCE LISTING (14 sequences)

SEQ ID NO: 1 - protein, 278 aa, Artificial Sequence
  recombinant Plasmodium Falciparum circumsporozoite polypeptide sequence
YGSSSNTRVLNELNYDNAGTNLYNELEMNYYGKQENWYSLKKNSRSLGENDDGNNEDNEKLRKPKHKKLKQPADGNPDPNANPNVDPNANPNVDPNANPNVDPNANPNANPNANPNANPNANPNANPNANPNANPNANPNANPNANPNANPNANPNANPNANPNANPNKNNQGNGQGHNMPNDPNRNVDENANANSAVKNNNNEEPSDKHIKEYLNKIQNSLSTEWSPCSVTCGNGIQVRIKPGSANKPKDELDYANDIEKKICKMEKCSSVFNVVNS

SEQ ID NO: 2 - DNA, 834 bp, Artificial Sequence
  recombinant Plasmodium Falciparum circumsporozoite protein nucleic acid sequence
tacggctcttcttctaacactcgcgtgctgaatgaactgaattacgataacgctggcaccaacctgtataatgaactggaaatgaactattacggtaagcaggaaaactggtatagcctgaaaaagaacagccgcagcctgggtgaaaacgacgacggtaacaacgaggacaatgaaaaactgcgcaagcctaaacacaaaaagctgaaacagccggcggacggtaatccggatccaaacgcaaacccgaatgtggatccgaacgccaatccgaacgtggacccgaacgcgaacccaaacgttgatcctaacgccaacccgaacgctaaccctaacgccaacccaaacgcaaaccctaatgctaacccaaacgcgaacccgaacgcaaatccgaacgcgaaccctaacgctaaccctaacgcaaaccctaacgcaaacccaaacgccaaccctaacgcgaacccgaatgcgaatccgaacgctaatccaaatgctaacccgaacaaaaacaaccagggcaacggccagggtcacaatatgccgaacgatccgaatcgcaacgtggacgaaaatgctaatgctaacagcgcagtgaaaaacaataataacgaggagccgagcgataagcacatcaaagaatatctgaacaagatccagaatagcctgtccaccgaatggagcccgtgctctgtcacgtgcggtaacggcattcaagttcgtatcaaaccaggtagcgccaacaagccgaaagacgaactggactacgcaaacgacattgagaaaaagatctgtaaaatggaaaaatgcagctctgtctttaacgtcgttaactcc

SEQ ID NO: 3 - DNA, 33 bp, Escherichia coli
  misc_feature: E. coli derived N terminal 6X-His tag nucleotide sequence derived from E. coli vector
atggcacaccatcatcatcatcatcccgggatg

SEQ ID NO: 4 - DNA, 36 bp, Escherichia coli
  misc_feature: E. Coli derived C-terminal 6XHIS tag nucleotide sequence derived from E. coli vector
ggcggccgcctcgagcaccaccaccaccaccactga

SEQ ID NO: 5 - DNA, 902 bp, Artificial Sequence
  rCS/D; recombinant Plasmodium Falciparum circumsporozoite protein nucleic acid sequence with 19 NANP repeats and 3 NVDP repeats, and including N and C terminal 6X HIS tags
atggcacaccatcatcatcatcatcccgggatgtacggctcttcttctaacactcgcgtgctgaatgaactgaattacgataacgctggcaccaacctgtataatgaactggaaatgaactattacggtaagcaggaaaactggtatagcctgaaaaagaacagccgcagcctgggtgaaaacgacgacggtaacaacgaggacaatgaaaaactgcgcaagcctaaacacaaaaagctgaaacagccggcggacggtaatccggatccaaacgcaaacccgaatgtggatccgaacgcaatccgaacgtggacccgaacgcgaacccaaacgttgatcctaacgccaacccgaacgctaaccctaacgccaacccaaacgcaaaccctaatgctaacccaaacgcgaacccgaacgcaaatccgaacgcgaaccctaacgctaaccctaacgcaaaccctaacgcaaacccaaacgccaaccctaacgcgaacccgaatgcgaatccgaacgctaatccaaatgctaacccgaacaaaaacaaccagggcaacggccagggtcacaatatgccgaacgatccgaatcgcaacgtggacgaaaatgctaatgctaacagcgcagtgaaaaacaataataacgaggagccgagcgataagcacatcaaagaatatctgaacaagatccagaatagcctgtccaccgaatggagcccgtgctctgtcacgtgcggtaacggcattcaagttcgtatcaaaccaggtagcgccaacaagccgaaagacgaactggactacgcaaacgacattgagaaaaagatctgtaaaatggaaaaatgcagctctgtctttaacgtcgttaactccggcggccgcctcgagcaccaccaccaccaccactga

SEQ ID NO: 6 - protein, 11 aa, Escherichia coli
  MISC_FEATURE: N-terminal 6X HIS tag polypeptide sequence derived from E. coli vector
MAHHHHHHPGM

SEQ ID NO: 7 - protein, 11 aa, Escherichia coli
  MISC_FEATURE: C-terminal 6X HIS tag polypeptide sequence derived from E. coli vector
GGRLEHHHHHH

SEQ ID NO: 8 - protein, 300 aa, Artificial Sequence
  rCS/D; recombinant Plasmodium Falciparum circumsporozoite polypeptide sequence including an N- and C-terminal E. Coli derived 6X HIS tags and Tyr26 start amino acid of CSP
MAHHHHHHPGMYGSSSNTRVLNELNYDNAGTNLYNELEMNYYGKQENWYSLKKNSRSLGENDDGNNEDNEKLRKPKHKKLKQPADGNPDPNANPNVDPNANPNVDPNANPNVDPNANPNANPNANPNANPNANPNANPNANPNANPNANPNANPNANPNANPNANPNANPNANPNANPNKNNQGNGQGHNMPNDPNRNVDENANANSAVKNNNNEEPSDKHIKEYLNKIQNSLSTEWSPCSVTCGNGIQVRIKPGSANKPKDELDYANDIEKKICKMEKCSSVFNVVNSGGRLEHHHHHH

SEQ ID NO: 9 - protein, 281 aa, Artificial Sequence
  rCS/A- recombinant Plasmodium Falciparum circumsporozoite polypeptide sequence with 18 NANP repeats and Gln21 starting amino acid and an N-terminal 6X HIS tag
MAHHHHHHPGGSQEYQCYGSSSNTRVLNELNYDNAGTNLYNELEMNYYGKQENWYSLKKNSRSLGENDDGNNEDNEKLRKPKHKKLKQPADGNPNANPNANPNANPNANPNANPNANPNANPNANPNANPNANPNANPNANPNANPNANPNANPNANPNANPNANPNKNNQGNGQGHNMPNDPNRNVDENANANSAVKNNNNEEPSDKHIKEYLNKIQNSLSTEWSPCSVTCGNGIQVRIKPGSANKPKDELDYANDIEKKICKMEKCSSVFNVVNSSIGL

SEQ ID NO: 10 - protein, 276 aa, Artificial Sequence
  rCS/B- recombinant Plasmodium Falciparum circumsporozoite polypeptide sequence with 18 NANP repeats and Tyr26 start amino acid and an N-terminal 6X HIS tag
MAHHHHHHPGGSYGSSSNTRVLNELNYDNAGTNLYNELEMNYYGKQENWYSLKKNSRSLGENDDGNNEDNEKLRKPKHKKLKQPADGNPNANPNANPNANPNANPNANPNANPNANPNANPNANPNANPNANPNANPNANPNANPNANPNANPNANPNANPNKNNQGNGQGHNMPNDPNRNVDENANANSAVKNNNNEEPSDKHIKEYLNKIQNSLSTEWSPCSVTCGNGIQVRIKPGSANKPKDELDYANDIEKKICKMEKCSSVFNVVNSSIGL

SEQ ID NO: 11 - protein, 228 aa, Artificial Sequence
  rCS/C- recombinant Plasmodium Falciparum circumsporozoite polypeptide with 5 NANP repeats and 2 NVDP repeats and Tyr26 start amino acid and a N-terminal 6X HIS tag sequence
MAHHHHHHPGYGSSSNTRVLNELNYDNAGTNLYNELEMNYYGKQENWYSLKKNSRSLGENDDGNNEDNEKLRKPKHKKLKQPADGNPDPNANPNVDPNANPNVDPNANPNANPNANPNKNNQGNGQGHNMPNDPNRNVDENANANSAGKNNNNEEPSDKHIKEYLNKIQNSLSTEWSPCSVTCGNGIQVRIKPGSANKPKDELDYANDIEKKICKMEKCSSVFNVVNS

SEQ ID NO: 12 - protein, 369 aa, Artificial Sequence
  rCS/E- recombinant Plasmodium Falciparum circumsporozoite polypeptide with 38 NANP repeats and 4 NVDP repeats and Tyr26 start amino acid and a N-terminal 6X HIS tag sequence
MAHHHHHHPGMYGSSSNTRVLNELNYDNAGTNLYNELEMNYYGKQENWYSLKKNSRSLGENDDGNNEDNEKLRKPKHKKLKQPADGNPDPNANPNVDPNANPNVDPNANPNVDPNANPNANPNANPNANPNANPNANPNANPNANPNANPNANPNANPNANPNANPNANPNANPNANPNANPNVDPNANPNANPNANPNANPNANPNANPNANPNANPNANPNANPNANPNANPNANPNANPNANPNANPNANPNANPNKNNQGNGQGHNMPNDPNRNVDENANANSAVKNNNNEEPSDKHIKEYLNKIQNSLSTEWSPCSVTCGNGIQVRIKPGSANKPKDELDYANDIEKKICKMEKCSSVFNVVNS

SEQ ID NO: 13 - protein, 4 aa, Artificial Sequence
  Repeat sequence derived from P. falciparum CSP
NANP

SEQ ID NO: 14 - protein, 4 aa, Artificial Sequence
  Repeat sequence derived from P. falciparum CSP
NVDP